European Patent Application EP 4 480 489 A1, published December 25, 2024. Title: COMPOSITION. Applicant: kyron.bio SAS. Application EP. The sequence listing filed with the application follows.

SEQUENCE LISTING (22 sequences)

SEQ ID NO: 1 - DNA, 69 bp, synthetic construct
  source 1..69: mol_type = other DNA
cgcgtccgtgcgttgttcgtgaaacatacgcgtaccggaaatcccctcgtggattctgtggctgagcat

SEQ ID NO: 2 - DNA, 120 bp, synthetic construct
  source 1..120: mol_type = other DNA
aaacctacagcgtaccgcgtccgtgcgttgttcgtgaaacatacgcgtaccggaaatcccctcgtggattctgtggctgagcatcggccgacgactgccggggcgtatctgcgctacttt

SEQ ID NO: 3 - DNA, 120 bp, synthetic construct
  source 1..120: mol_type = other DNA; note = DNA sequence of active region of TbSTT3A (CHO optimised)
aagcctaccgcctacagagtgcgggccctgtttgtgaagcacaccagaaccggcaatcctctggtggactctgtggccgagcatagacctacaaccgctggcgcctacctgcggtacttt

SEQ ID NO: 4 - DNA, 120 bp, synthetic construct
  source 1..120: mol_type = other DNA
aggccgttttcttctcgtgtccgtgcgttgttcgtgaaacatacgcgtaccggaaatcccctcgtggattctgtggctgagcaccatccggcgtcgaatgatgatttctttggttacctt

SEQ ID NO: 5 - DNA, 120 bp, synthetic construct
  source 1..120: mol_type = other DNA
cggcctttcagctctagagtgcgggccctgtttgtgaagcacaccagaaccggcaatcctctggtggactctgtggccgagcaccatcctgcctctaacgacgacttcttcggctacctg

SEQ ID NO: 6 - DNA, 120 bp, synthetic construct
  source 1..120: mol_type = other DNA
aggtcgttttcttctcgtgtccgtgcgttgttcgtgaaacatacgcgtaccggaaatcccctcgtggattctgtggctgagcatcggccgacgactgccggggccttcctacgtcatctt

SEQ ID NO: 7 - DNA, 120 bp, synthetic construct
  source 1..120: mol_type = other DNA
cggtccttcagctctagagtgcgggccctgtttgtgaagcacaccagaaccggcaatcctctggtggactctgtggccgagcatcggcctacaacagctggcgcctttctgagacatctg

SEQ ID NO: 8 - DNA, 2406 bp, Trypanosoma brucei
  source 1..2406: mol_type = other DNA
atgacgaaaggtgggaaagtagctgtgactaagggctcagcacagagtgatggtgctggtgagggagggatgagtaaggccaagtcatccactacgttcgtcgccactggcggtggttctttgcctgcctgggcgctaaaggctgtaagcacgattgtgagtgcagtgattcttatatactctgtccatcgtgcttacgatatacgacttacttctgtccgtctttatggtgagcttattcacgagttcgacccttggttcaattaccgtgcaacgcagtacctcagcgacaacgggtggcgtgcttttttccaatggtacgactacatgagctggtacccgcttggccgaccggtgggcacaaccatcttccccggaatgcagcttaccggtgtagccattcatcgtgtgctggaaatgctcgggcgaggtatgtccatcaacaatatctgtgtgtacattcctgcatggttcggtagtattgccactgtgttggctgctctcattgcgtacgaatcatctaattcgctcagtgtcatggcgtttactgcgtactttttttccatcgtacctgcacacctgatgcgatcaatggctggtgaatttgacaatgagtgtgttgcaatggcggcgatgcttctgacgttctacatgtgggtacgatcgttacgcagctcaagttcgtggcccattggcgctttagctggtgtggcatacgggtacatggtgtccacgtggggtggttatattttcgtgctgaacatggtagccttccacgcttctgtatgtgtactgcttgattgggctcgtgggatatacagcgtcagtttgctgagggcgtattcactgttttttgtcattggcactgcccttgcgatttgcgtaccgccagtggagtggacgcccttccggtcgctggagcaactgacagcattgtttgtcttcgttttcatgtgggcactccactactcggaatacctgcgtgagcgtgcccgagcgcccattcactcttctaaagcacttcagatccgtgcccgcattttcatgggcaccctctccttgctgttgattgtggcaagtttgcttgccccgttcggattcttcaaacctacagcgtaccgcgtccgtgcgttgttcgtgaaacatacgcgtaccggaaatcccctcgtggattctgtggctgagcatcggccgacgactgccggggcgtatctgcgctactttcatgtttgttaccctctttgggggtgcggtgggctctctatgttggtattcatgaaaaaggaccgctggcgcgccattgtttttcttgcttcactttccactgttacgatgtatttcagcgcccgtatgtcgcgattacttctgttagcgggtcccgcagcaacggcttgcgccggcatgttcataggggggctttttgatctggcgctgtcacagtttggtgatttgcatagcccaaaagatgcctccggcgattccgatcccgcgggagggtcgaagcgggcaaagggcaaagttgttaatgagccttccaaaagagccatctttagtcaccgctggtttcaacgtttagtgcaatcgttgcccgtcccgctacgacgtggtatcgcggttgtggtgctcgtatgtctcttcgccaatcccatgagacactcattcgaaaagtcctgcgagaaaatggcacatgcactttcatctccaaggatcattgccgtgactgatctacccaatggagagagagtcctcgccgatgattactacgtgtcgtacttgtggctgcgaaacaatacgcctgaagatgcccgtattctctcatggtgggactacgggtatcaaatcactggaattggcaatcgcacaacccttgcggacggtaacacatggagtcacaagcacatagcaactattgggaagatgcttacatcccctgtgaaggagtcacatgctcttatacgccatctcgctgattatgtgctgatatgggccggtgaggatcggggcgatttacttaaatcgccacacatggctcggataggcaacagtgtatatcgcgatatgtgttcagaagacgatcctagatgcaggcagttcggctttgagggaggtgacctcaataagcctacgcctatgatgcagcggtccctattatacaatctgcacaggtttggtacggatggcgggaagacacaactggataagaacatgtttcagctcgcctacgtgtcaaagtatggtttggtgaagatctacaaggtggtgaatgtgagtgaagagagcaaggcgtgggtcgcagacccaaagaaccgcgtatgcgacccgcccggatcttggatatgcgccggccagtacccgccagcgaaggagatccaagacatgttagcgaagcggttccattacgaatga

SEQ ID NO: 9 - DNA, 2406 bp, synthetic construct
  source 1..2406: mol_type = other DNA
atgaccaaaggcggaaaagtggctgtgaccaagggctctgctcagtctgatggtgctggcgaaggcggcatgtctaaggccaagtcctctaccaccttcgtggctaccggcggaggatctttgcctgcttgggctctgaaggccgtgtccaccattgtgtctgccgtgatcctgatctactccgtgcaccgggcctacgacatcaggctgacatctgtcagactgtacggcgagctgatccacgagttcgacccctggttcaactaccgggctacccagtacctgtccgataatggctggcgggccttcttccagtggtacgactatatgtcctggtatcccctgggcagacccgtgggcaccacaatctttccaggcatgcagctgacaggcgtggccatccatagagtgctggaaatgctcggcagaggcatgtccatcaacaacatctgcgtgtacatccccgcttggtttggctctatcgccaccgttctggccgctctgatcgcctacgagtcctccaactctctgtccgtgatggccttcaccgcctactttttctccatcgtgcccgctcacctgatgcggtctatggccggcgagttcgataacgagtgtgtggccatggctgccatgctgctgaccttctatatgtgggtccgaagcctgcggtcctcctccagttggcctattggagctttggccggcgtggcctacggctacatggtttctacctggggcggctacatcttcgtgctgaacatggtggccttccacgcctctgtgtgcgtgctgttggattgggccagaggcatctacagcgtgtccctgctgagagcctacagcctgttcttcgtgatcggcacagccctggccatctgtgtgccacctgttgagtggacccctttcagatccctggaacagctgaccgctctgttcgtgtttgtgttcatgtgggccctgcactactccgagtacctgagagagagagccagggctcccatccactcttctaaggccctgcagatccgggccagaatcttcatgggcaccctgagcctgctgctgatcgtggcttctctgctggcccctttcggcttctttaagcctaccgcctacagagtgcgggccctgtttgtgaagcacaccagaaccggcaatcctctggtggactctgtggccgagcatagacctacaaccgctggcgcctacctgcggtactttcacgtgtgctatcctctgtggggctgtggcggactgtccatgctggtgttcatgaagaaagaccggtggcgggccatcgtgtttctggctagtctgtccaccgtgaccatgtacttcagcgcccggatgtccagactgctgctgttggctggacctgccgctacagcttgtgccggcatgtttatcggcggcctgttcgatctggccctgtctcagtttggcgacctgcactctcctaaggacgcctctggcgactctgatcctgctggcggatccaagcgcgctaagggcaaagtggtcaacgagccttccaagagagccatcttctctcaccggtggttccagcggctggtgcagtctcttccagttcctctgagaagaggaatcgccgtggtggtgctcgtgtgcctgttcgccaatcctatgcggcactccttcgagaagtcctgcgagaaaatggcccacgctctgagcagccctcggatcattgctgtgaccgatctgcccaacggcgagcgagttctggctgacgattactacgtgtcctacctgtggctgcggaacaacacccctgaggacgccagaatcctgtcttggtgggattacggctaccagatcaccggcatcggcaacagaaccacactggccgatggcaacacatggtcccacaagcacattgccaccatcggcaagatgctgacctctcctgtgaaagagtctcacgccctgatcagacacctggccgactacgtgttgatctgggctggggaagatcggggcgatctgctgaagtctcctcacatggccaggatcggcaactctgtgtaccgggacatgtgctccgaggacgaccctagatgtcggcagttcggatttgaaggcggcgacctgaacaagcccacacctatgatgcagagatccctgctgtacaacctgcacagattcggcaccgatggcggcaagacccagctggacaagaacatgtttcagctggcctacgtcagcaaatacggcctggtcaagatctacaaggtcgtgaacgtgtccgaggaatccaaggcctgggtcgccgatcctaagaatagagtgtgcgaccctcctggctcctggatctgtgctggacagtaccctcctgccaaagaaatccaggacatgctggccaagcggttccactacgaatga

SEQ ID NO: 10 - DNA, 2466 bp, Trypanosoma brucei
  source 1..2466: mol_type = other DNA
atgacgaaaggtgggaaagtagctgtgactaagggctcagcacagagtgatggtgctggtgagggagggatgagtaaggccaagtcatccactacgttcgtcgccactggcggtggttctttgcctgcctgggcgctaaaggctgtaagcacggttgtgagtgcagtgattcttatatactctgtccatcgtgcttacgatatacgacttacttctgtccgtctttatggtgagcttattcacgagttcgacccttggttcaattaccgtgcaacgcagtacctcagcgacaacgggtggcgtgcttttttccaatggtacgactacatgagctggtacccgcttggccgaccggtgggcacaaccatcttccccggaatgcagcttaccggtgtagccattcatcgtgtgctggaaatgctcgggcgaggtatgtccatcaacaatatctgtgtgtacattcctgcatggttcggtagtattgccactgtgttggctgctctcattgcgtacgaatcatctaattcgctcagtgtcatggcgtttactgcgtactttttttccatcgtacctgcacacctgatgcgatcaatggctggtgaatttgacaatgagtgtgttgcaatggcggcgatgcttctgacgttctacatgtgggtacgatcgttacgcagctcaagttcgtggcccattggcgctttagctggtgtggcatacgggtacatggtgtccacgtggggtggttatattttcgtgctgaacatggtagccttccacgcttctgtatgtgtactgcttgattgggctcgtgggacatacagcgtcagtttgctgagggcgtattcactgttttttgtcattggcactgcccttgcgatttgcgtaccaccagtggagtggacgcccttccggtcgctggagcaactgacagcattgtttgtcttcgttttcatgtgggcactccactactcggaatacctgcgtgagcgtgcccgagcgcccattcactcttctaaagcacttcagatccgtgcccgcattttcatgggcaccctctccttgctgttgattgtagctatctacctattttcgacaggatacttcaggccgttttcttctcgtgtccgtgcgttgttcgtgaaacatacgcgtaccggaaatcccctcgtggattctgtggctgagcaccatccggcgtcgaatgatgatttctttggttaccttcatgtatgttacaacggctggataattggctttttcttcatgtccgtgtcgtgctttttccattgtacaccgggaatgtcgttcctgctgttgtactctatacttgcgtactacttctctctcaagatgagtcgtctgctgttactttctgcacctgtggcttccatactcactggctatgttgtgggatctattgttgacctcgcagcagattgtttcgccgcttccggaacagagcacgccgacagtaaggagcatcaagggaaagcccgtggtaagggacagaaggaacaaatcactgtcgagtgtgggtgccataatcccttctacaaattatggtgcaattcattttcctcccgcctggtagttggtaagttttttgtcgttgttgtcctttccatctgtggacccacatttcttgggtctaacttccggatatattctgagcaattcgcagacagcatgtcgagcccccagattataatgagggcaactgtcggtggacgacgagttatcttggatgattactacgtgtcgtacttgtggctgcgaaacaatacgcctgaagatgcccgtattctctcatggtgggactacgggtatcaaatcactggaattggcaatcgcacaacccttgcggatggtaacacatggaatcacgagcacatagcaactattgggaagatgcttacatcccctgtgaaggagtcacatgctcttatacgccatctcgctgattatgtgctgatatgggccggttatgatggcagcgatttacttaaatcgccacacatggctcggataggcaacagtgtatatcgcgatatatgctcagaggatgatccgctgtgtacgcagttcgggttttatagtggtgacttcagtaaacctacgcctatgatgcagcggtccctattatacaatctgcacaggtttggtacggatggcgggaagacacaactggataagaacatgtttcagctcgcctacgtgtcaaagtatggtttggtgaagatctacaaggtgatgaatgtgagtgaagagagcaaggcgtgggttgcagacccaaagaaccgtaagtgcgatgcacctggatcttggatatgcaccggccagtacccgccagcgaaggagatccaagacatgttagcgaagaggattgactacgaacaactcgaggatttcaaccgccgcaatcgaagtgacgcttattatcgtgcgtatatgcgtcagatgggttag

SEQ ID NO: 11 - DNA, 2466 bp, synthetic construct
  source 1..2466: mol_type = other DNA
atgaccaaaggcggaaaagtggctgtgaccaagggctctgctcagtctgatggtgctggcgaaggcggcatgtctaaggccaagtcctctaccaccttcgtggctaccggcggaggatctttgcctgcttgggctctgaaggccgtgtccacagtggtgtctgccgtgatcctgatctactctgtgcaccgggcctacgacatccggctgacatctgtcagactgtacggcgagctgatccacgagttcgacccctggttcaactaccgggctacccagtacctgtccgataatggctggcgggccttcttccagtggtacgactatatgtcctggtatcccctgggcagacccgtgggcaccacaatctttccaggcatgcagctgacaggcgtggccatccatagagtgctggaaatgctcggcagaggcatgtccatcaacaacatctgcgtgtacatccccgcttggtttggctctatcgccaccgttctggccgctctgatcgcctacgagtcctccaactctctgtccgtgatggccttcaccgcctactttttctccatcgtgcccgctcacctgatgcggtctatggccggcgagttcgataacgagtgtgtggccatggctgccatgctgctgaccttctatatgtgggtccgaagcctgcggtcctcctccagttggcctattggagctttggccggcgtggcctacggctacatggtttctacctggggcggctacatcttcgtgctgaacatggtggccttccacgcctctgtgtgcgtgctgttggattgggctagaggcacctactccgtgtctctgctgagagcctacagcctgttcttcgtgatcggcacagccctggccatctgtgtgccacctgttgagtggacccctttcagatccctggaacagctgaccgctctgttcgtgtttgtgttcatgtgggccctgcactactccgagtacctgagagagagagccagggctcccatccactcttctaaggccctgcagatccgggccagaatcttcatgggcacactgtccctgctgctgatcgtggctatctacctgttctccaccggctacttccggcctttcagctctagagtgcgggccctgtttgtgaagcacaccagaaccggcaatcctctggtggactctgtggccgagcaccatcctgcctctaacgacgacttcttcggctacctgcacgtgtgctacaacggctggatcatcggctttttctttatgtctgtgtcctgcttcttccactgtacccctggcatgtcctttctgctgctgtactccatcctggcctactacttcagcctgaagatgtctagactgctgctgctctctgcccctgtggcctctatcctgaccggatatgtcgtgggcagcatcgtggatctggccgccgactgttttgctgcttctggcaccgagcacgccgactccaaagagcatcagggcaaagccagaggcaagggccagaaagagcagatcaccgtcgagtgcggctgtcacaaccccttctacaagctgtggtgcaactccttctcctctcggctggtcgtgggaaagttctttgtggtggtggtgctgtctatctgcggccctaccttcctgggctccaacttcagaatctacagcgagcagttcgccgacagcatgtctagccctcagatcatcatgagagccaccgtcggcggcagaagagtgatcctggacgactactacgtgtcctacctgtggctgcggaacaacacccctgaggacgccagaatcctgtcttggtgggattacggctaccagatcacaggcatcggcaacagaaccacactggccgatggcaacacctggaaccacgagcacattgccaccatcggcaagatgctgacctctcctgtgaaagagtctcacgccctgatcagacacctggccgactacgtgctgatctgggctggctacgatggctccgacctgctgaagtctcctcacatggccaggatcggcaattccgtgtaccgggacatctgctccgaggacgatcctctgtgtacccagttcggcttctactccggcgacttctccaagcctacacctatgatgcagcggagcctgctgtacaacctgcacagatttggcaccgatggcggcaagacccagctggacaagaacatgtttcagctggcctacgtcagcaaatacggcctggtcaagatctacaaagtgatgaacgtgtccgaggaatccaaggcctgggtcgccgatcctaagaaccggaagtgtgacgctcctggcagctggatctgcaccggacaataccctccagccaaagaaatccaggacatgctggccaagcggatcgactacgagcagctggaagatttcaaccggcggaacagatccgacgcctactaccgcgcttacatgcggcagatgggatga

SEQ ID NO: 12 - DNA, 2466 bp, Trypanosoma brucei
  source 1..2466: mol_type = other DNA
atgacgaaaggtgggaaagtagctgtgactaagggctcagcacagagtgatggtgctggtgagggagggatgagtaaggccaagtcatccactacgttcgtcgccactggcggtggttctttgcctgcctgggcgctaaaggctgtaagcacggttgtgagtgcagtgattcttatatactctgtccatcgtgcttacgatatacgacttacttctgtccgtctttatggtgagcttattcacgagttcgacccttggttcaattaccgtgcaacgcagtacctcagcgacaacgggtggcgtgcttttttccaatggtacgactacatgagctggtacccgcttggccgaccggtgggcacaaccatcttccccggaatgcagcttaccggtgtagccattcatcgtgtgctggaaatgctcgggcgaggtatgtccatcaacaatatctgtgtgtacattcctgcatggttcggtagtattgccactgtgttggctgctctcattgcgtacgagtcatctaattcgctcagtgtcatggcgtttactgcgtactttttttccatcgtacctgcacacctgatgcgatcaatggctggtgaatttgacaatgagtgtgttgcaatggcggcgatgcttctgacgttctacatgtgggtacgatcgttacgcagctcaagttcgtggcccattggcgctttagctggtgtggcatacgggtacatggtgtccacgtggggtggttatattttcgtgctgaacatggtagccttccacgcttctgtatgtgtactgcttgattgggctcgtgggacatacagcgtcagtttgctgagggcgtattcactgttttttgtcattggcactgcccttgcgatttgcgtaccaccagtggagtggacgcccttccggtcgctggagcaactgacagcattgtttgtcttcgttttcatgtgggcactccactactcggaatacctgcgtgagcgtgcccgagcgcccattcactcttctaaagcacttcagatccgtgcccgcattttcatgggcaccctctccttgctgttgattgtggctatctacctattttcgacaggatacttcaggtcgttttcttctcgtgtccgtgcgttgttcgtgaaacatacgcgtaccggaaatcccctcgtggattctgtggctgagcatcggccgacgactgccggggccttcctacgtcatcttcatgtgtgttacaacggctggataattggctttttcttcatgtccgtgtcgtgctttttccattgtacaccgggaatgtcgttcctgctgttgtactctatacttgcgtactacttctctctcaagatgagtcgtctgctgttactttctgcacctgtggcttccatactcactggctatgttgtgggatctattgttgacctcgcagcagattgtttcgccgcttccggaacagagcacgccgacagtaaggagcatcaagggaaagcccgtggtaagggacaaaagagacaaatcactgtcgagtgtgggtgccataatcccttctacaaattatggtgcaattcattttcctcccgcctggtagttggtaagttttttgtcgttgttgtcctttccatctgtggacccacatttcttgggtctgagtttagggctcattgcgaacgtttctccgtaagtgttgctaatccgcgtattatatcgagtattaggcactccggtaagttggttcttgccgatgattactacgtgtcgtacttgtggctgcgaaacaatacgcctgaagatgcccgtattctctcatggtgggactacgggtatcaaatcactggaattggcaatcgcacaacccttgcggacggtaacacatggaatcacgagcacatagcaactattgggaagatgcttacatcccctgtgaaggagtcacatgctcttatacgccatctcgctgattatgtgctgatatgggccggtgaggatcggggcgatttacgtaagtcacggcatatggctcggataggcaacagtgtatatcgcgatatgtgttcagaagacgatccgctgtgtacgcagttcgggttttatagtggtgacttcaataaacctacgcctatgatgcagcggtccctattatacaatctgcacaggtttggtacggatggcgggaagacacaactggataagaacatgtttcagctcgcctacgtgtcaaagtatggtttggtgaagatctacaaggtgatgaatgtgagtgaagagagcaaggcgtgggttgcagacccaaagaaccgtaagtgcgatgcacctggatcttggatatgcgccggccagtacccgccagcgaaggagatccaagacatgttagcgaagaggattgactacgaacaactcgaggatttcaatcgccgcaatcgaagtgacgcttattatcgtgcgtatatgcgtcagatgggttag

SEQ ID NO: 13 - DNA, 2466 bp, synthetic construct
  source 1..2466: mol_type = other DNA
atgaccaaaggcggaaaagtggctgtgaccaagggctctgctcagtctgatggtgctggcgaaggcggcatgtctaaggccaagtcctctaccaccttcgtggctaccggcggaggatctttgcctgcttgggctctgaaggccgtgtccacagtggtgtctgccgtgatcctgatctactctgtgcaccgggcctacgacatccggctgacatctgtcagactgtacggcgagctgatccacgagttcgacccctggttcaactaccgggctacccagtacctgtccgataatggctggcgggccttcttccagtggtacgactatatgtcctggtatcccctgggcagacccgtgggcaccacaatctttccaggcatgcagctgacaggcgtggccatccatagagtgctggaaatgctcggcagaggcatgtccatcaacaacatctgcgtgtacatccccgcttggtttggctctatcgccaccgttctggccgctctgatcgcctacgagtcctccaactctctgtccgtgatggccttcaccgcctactttttctccatcgtgcccgctcacctgatgcggtctatggccggcgagttcgataacgagtgtgtggccatggctgccatgctgctgaccttctatatgtgggtccgaagcctgcggtcctcctccagttggcctattggagctttggccggcgtggcctacggctacatggtttctacctggggcggctacatcttcgtgctgaacatggtggccttccacgcctctgtgtgcgtgctgttggattgggctagaggcacctactccgtgtctctgctgagagcctacagcctgttcttcgtgatcggcacagccctggccatctgtgtgccacctgttgagtggacccctttcagatccctggaacagctgaccgctctgttcgtgtttgtgttcatgtgggccctgcactactccgagtacctgagagagagagccagggctcccatccactcttctaaggccctgcagatccgggccagaatcttcatgggcacactgtccctgctgctgatcgtggctatctacctgttctccaccggctacttccggtccttcagctctagagtgcgggccctgtttgtgaagcacaccagaaccggcaatcctctggtggactctgtggccgagcatcggcctacaacagctggcgcctttctgagacatctgcacgtgtgctacaacggctggatcatcggctttttctttatgtctgtgtcctgcttcttccactgtacccctggcatgtcctttctgctgctgtactccatcctggcctactacttcagcctgaagatgtctagactgctgctgctctctgcccctgtggcctctatcctgaccggatatgtcgtgggcagcatcgtggatctggccgccgactgttttgctgcttctggcaccgagcacgccgactccaaagagcatcagggcaaagccagaggcaagggccagaaaagacagatcaccgtggaatgcggctgtcacaaccccttctacaagctgtggtgcaactccttctcctctcggctggtcgtgggaaagttctttgtggtggtggtgctgtctatctgcggccctacctttctgggctccgagtttagagcccactgcgagagattctccgtgtccgtggccaatcctcggatcatctcctccatccggcactccggaaagctggtcctggccgacgactactacgtgtcctacctgtggctgcggaacaacacccctgaggacgccagaatcctgtcttggtgggattacggctaccagatcacaggcatcggcaacagaaccacactggccgatggcaacacctggaaccacgagcacattgccaccatcggcaagatgctgacctctcctgtgaaagagtctcacgccctgatccggcacctggccgattatgtgttgatctgggctggcgaggaccggggcgatctgagaaagtccagacacatggctcggatcggcaactccgtgtaccgggacatgtgctctgaggacgaccctctgtgtacccagttcggcttctactccggcgacttcaacaagcccacacctatgatgcagcggagcctgctgtacaacctgcacagatttggcaccgacggcggcaagacccagctggacaagaacatgtttcagctggcctacgtcagcaaatacggcctggtcaagatctacaaagtgatgaacgtgtccgaggaatccaaggcctgggtcgccgatcctaagaaccggaagtgtgacgctcctggctcctggatctgtgccggacaataccctcctgccaaagaaatccaggacatgctggccaagcggatcgactacgagcagctggaagatttcaaccggcggaacagaagcgacgcctactaccgcgcttacatgcggcagatgggatga

SEQ ID NO: 14 - protein, 42 aa, synthetic construct
FFKPTAYRVRALFVKHTRTGNPLVDSVAEHRPTTAGAYLRYF

SEQ ID NO: 15 - protein, 42 aa, synthetic construct
YFRPFSSRVRALFVKHTRTGNPLVDSVAEHHPASNDDFFGYL

SEQ ID NO: 16 - protein, 42 aa, synthetic construct
YFRPFSSRVRALFVKHTRTGNPLVDSVAEHRPTTAGAFLRHL

SEQ ID NO: 17 - protein, 801 aa, Trypanosoma brucei
MTKGGKVAVTKGSAQSDGAGEGGMSKAKSSTTFVATGGGSLPAWALKAVSTIVSAVILIYSVHRAYDIRLTSVRLYGELIHEFDPWFNYRATQYLSDNGWRAFFQWYDYMSWYPLGRPVGTTIFPGMQLTGVAIHRVLEMLGRGMSINNICVYIPAWFGSIATVLAALIAYESSNSLSVMAFTAYFFSIVPAHLMRSMAGEFDNECVAMAAMLLTFYMWVRSLRSSSSWPIGALAGVAYGYMVSTWGGYIFVLNMVAFHASVCVLLDWARGIYSVSLLRAYSLFFVIGTALAICVPPVEWTPFRSLEQLTALFVFVFMWALHYSEYLRERARAPIHSSKALQIRARIFMGTLSLLLIVASLLAPFGFFKPTAYRVRALFVKHTRTGNPLVDSVAEHRPTTAGAYLRYFHVCYPLWGCGGLSMLVFMKKDRWRAIVFLASLSTVTMYFSARMSRLLLLAGPAATACAGMFIGGLFDLALSQFGDLHSPKDASGDSDPAGGSKRAKGKVVNEPSKRAIFSHRWFQRLVQSLPVPLRRGIAVVVLVCLFANPMRHSFEKSCEKMAHALSSPRIIAVTDLPNGERVLADDYYVSYLWLRNNTPEDARILSWWDYGYQITGIGNRTTLADGNTWSHKHIATIGKMLTSPVKESHALIRHLADYVLIWAGEDRGDLLKSPHMARIGNSVYRDMCSEDDPRCRQFGFEGGDLNKPTPMMQRSLLYNLHRFGTDGGKTQLDKNMFQLAYVSKYGLVKIYKVVNVSEESKAWVADPKNRVCDPPGSWICAGQYPPAKEIQDMLAKRFHYE

SEQ ID NO: 18 - protein, 821 aa, Trypanosoma brucei
MTKGGKVAVTKGSAQSDGAGEGGMSKAKSSTTFVATGGGSLPAWALKAVSTVVSAVILIYSVHRAYDIRLTSVRLYGELIHEFDPWFNYRATQYLSDNGWRAFFQWYDYMSWYPLGRPVGTTIFPGMQLTGVAIHRVLEMLGRGMSINNICVYIPAWFGSIATVLAALIAYESSNSLSVMAFTAYFFSIVPAHLMRSMAGEFDNECVAMAAMLLTFYMWVRSLRSSSSWPIGALAGVAYGYMVSTWGGYIFVLNMVAFHASVCVLLDWARGTYSVSLLRAYSLFFVIGTALAICVPPVEWTPFRSLEQLTALFVFVFMWALHYSEYLRERARAPIHSSKALQIRARIFMGTLSLLLIVAIYLFSTGYFRPFSSRVRALFVKHTRTGNPLVDSVAEHHPASNDDFFGYLHVCYNGWIIGFFFMSVSCFFHCTPGMSFLLLYSILAYYFSLKMSRLLLLSAPVASILTGYVVGSIVDLAADCFAASGTEHADSKEHQGKARGKGQKEQITVECGCHNPFYKLWCNSFSSRLVVGKFFVVVVLSICGPTFLGSNFRIYSEQFADSMSSPQIIMRATVGGRRVILDDYYVSYLWLRNNTPEDARILSWWDYGYQITGIGNRTTLADGNTWNHEHIATIGKMLTSPVKESHALIRHLADYVLIWAGYDGSDLLKSPHMARIGNSVYRDICSEDDPLCTQFGFYSGDFSKPTPMMQRSLLYNLHRFGTDGGKTQLDKNMFQLAYVSKYGLVKIYKVMNVSEESKAWVADPKNRKCDAPGSWICTGQYPPAKEIQDMLAKRIDYEQLEDFNRRNRSDAYYRAYMRQMG

SEQ ID NO: 19 - protein, 821 aa, Trypanosoma brucei
MTKGGKVAVTKGSAQSDGAGEGGMSKAKSSTTFVATGGGSLPAWALKAVSTVVSAVILIYSVHRAYDIRLTSVRLYGELIHEFDPWFNYRATQYLSDNGWRAFFQWYDYMSWYPLGRPVGTTIFPGMQLTGVAIHRVLEMLGRGMSINNICVYIPAWFGSIATVLAALIAYESSNSLSVMAFTAYFFSIVPAHLMRSMAGEFDNECVAMAAMLLTFYMWVRSLRSSSSWPIGALAGVAYGYMVSTWGGYIFVLNMVAFHASVCVLLDWARGTYSVSLLRAYSLFFVIGTALAICVPPVEWTPFRSLEQLTALFVFVFMWALHYSEYLRERARAPIHSSKALQIRARIFMGTLSLLLIVAIYLFSTGYFRSFSSRVRALFVKHTRTGNPLVDSVAEHRPTTAGAFLRHLHVCYNGWIIGFFFMSVSCFFHCTPGMSFLLLYSILAYYFSLKMSRLLLLSAPVASILTGYVVGSIVDLAADCFAASGTEHADSKEHQGKARGKGQKRQITVECGCHNPFYKLWCNSFSSRLVVGKFFVVVVLSICGPTFLGSEFRAHCERFSVSVANPRIISSIRHSGKLVLADDYYVSYLWLRNNTPEDARILSWWDYGYQITGIGNRTTLADGNTWNHEHIATIGKMLTSPVKESHALIRHLADYVLIWAGEDRGDLRKSRHMARIGNSVYRDMCSEDDPLCTQFGFYSGDFNKPTPMMQRSLLYNLHRFGTDGGKTQLDKNMFQLAYVSKYGLVKIYKVMNVSEESKAWVADPKNRKCDAPGSWICAGQYPPAKEIQDMLAKRIDYEQLEDFNRRNRSDAYYRAYMRQMG

SEQ ID NO: 20 - protein, 23 aa, synthetic construct
RVRALFVKHTRTGNPLVDSVAEH

SEQ ID NO: 21 - DNA, 69 bp, synthetic construct
  source 1..69: mol_type = other DNA
cgtgtccgtgcgttgttcgtgaaacatacgcgtaccggaaatcccctcgtggattctgtggctgagcac

SEQ ID NO: 22 - DNA, 69 bp, synthetic construct
  source 1..69: mol_type = other DNA
cgtgtccgtgcgttgttcgtgaaacatacgcgtaccggaaatcccctcgtggattctgtggctgagcat